European Patent Application EP 4 299 758 A1, published January 3, 2024. Title: 一种靶向富集核酸的探针. Applicant: 纳昂达（南京）生物科技有限公司. Application WO, filed July 14, 2022. The sequence listing filed with the application follows.

SEQUENCE LISTING (379 sequences)

SEQ ID NO: 1 - DNA, 120 bp, synthetic construct
  source 1..120: mol_type = other DNA
tgctgaaagctgtaccatacctgtctggtcttggctgaggtttcaatgaatggaatcccgtaactcttggccagttcgtgggcttgttttgtatcaactgtccttgttggcaaatcacac

SEQ ID NO: 2 - DNA, 120 bp, synthetic construct
  source 1..120: mol_type = other DNA
tttcaatgaatggaatcccgtaactcttggccagttcgtgggcttgttttgtatcaactgtccttgttggcaaatcacacttgtttcccactagcaccataggtacatcatccgagtctt

SEQ ID NO: 3 - DNA, 120 bp, synthetic construct
  source 1..120: mol_type = other DNA
gctattattgatggcaaatacacagaggaagccttcgcctgtcctcatgtattggtctctcatggcactgtactcttcttgtccagctgtatccagtatgtccaacaaacaggtttcacc

SEQ ID NO: 4 - DNA, 120 bp, synthetic construct
  source 1..120: mol_type = other DNA
attggtctctcatggcactgtactcttcttgtccagctgtatccagtatgtccaacaaacaggtttcaccatctataaccacttgttttctgtaagaatcctgggggtgtggagggtaag

SEQ ID NO: 5 - DNA, 120 bp, synthetic construct
  source 1..120: mol_type = other DNA
taccactgggcctcacctctatggtgggatcatattcatctacaaagtggttctggattagctggattgtcagtgcgcttttcccaacaccacctgctccaaccaccaccagtttgtact

SEQ ID NO: 6 - DNA, 120 bp, synthetic construct
  source 1..120: mol_type = other DNA
ctcacctctatggtgggatcatattcatctacaaagtggttctggattagctggattgtcagtgcgcttttcccaacaccacctgctccaaccaccaccagtttgtactcagtcatttca

SEQ ID NO: 7 - DNA, 120 bp, synthetic construct
  source 1..120: mol_type = other DNA
tttatttcagtgttacttacctgtcttgtctttgctgatgtttcaataaaaggaattccataacttcttgctaagtcctgagcctgttttgtgtctactgttctagaaggcaaatcacat

SEQ ID NO: 8 - DNA, 120 bp, synthetic construct
  source 1..120: mol_type = other DNA
tttcaataaaaggaattccataacttcttgctaagtcctgagcctgttttgtgtctactgttctagaaggcaaatcacatttatttcctactaggaccataggtacatcttcagagtcct

SEQ ID NO: 9 - DNA, 120 bp, synthetic construct
  source 1..120: mol_type = other DNA
agcctgttttgtgtctactgttctagaaggcaaatcacatttatttcctactaggaccataggtacatcttcagagtccttaactcttttaatttgttctctgggaaagaaaaaaaagtt

SEQ ID NO: 10 - DNA, 120 bp, synthetic construct
  source 1..120: mol_type = other DNA
agtattatttatggcaaatacacaaagaaagccctccccagtcctcatgtactggtccctcattgcactgtactcctcttgacctgctgtgtcgagaatatccaagagacaggtttctcc

SEQ ID NO: 11 - DNA, 120 bp, synthetic construct
  source 1..120: mol_type = other DNA
actggtccctcattgcactgtactcctcttgacctgctgtgtcgagaatatccaagagacaggtttctccatcaattactacttgcttcctgtaggaatcctgagaagggagaaacacag

SEQ ID NO: 12 - DNA, 120 bp, synthetic construct
  source 1..120: mol_type = other DNA
tttacctctattgttggatcatattcgtccacaaaatgattctgaattagctgtatcgtcaaggcactcttgcctacgccaccagctccaactaccacaagtttatattcagtcattttc

SEQ ID NO: 13 - DNA, 120 bp, synthetic construct
  source 1..120: mol_type = other DNA
gtccacaaaatgattctgaattagctgtatcgtcaaggcactcttgcctacgccaccagctccaactaccacaagtttatattcagtcattttcagcaggccttataataaaaataatga

SEQ ID NO: 14 - DNA, 120 bp, synthetic construct
  source 1..120: mol_type = other DNA
tttccaatggactattttagaagaaatggagctgtcacccacatcaagattcagaacactggtgattactatgacctgtatggaggggagaaatttgccactttggctgagttggtccag

SEQ ID NO: 15 - DNA, 120 bp, synthetic construct
  source 1..120: mol_type = other DNA
actggtgattactatgacctgtatggaggggagaaatttgccactttggctgagttggtccagtattacatggaacatcacgggcaattaaaagagaagaatggagatgtcattgagctt

SEQ ID NO: 16 - DNA, 120 bp, synthetic construct
  source 1..120: mol_type = other DNA
tcatgatgtttccttcgtaggtgttgactgcgatattgacgttcccaaaaccatccagatggtgcggtctcagaggtcagggatggtccagacagaagcacagtaccgatttatctatat

SEQ ID NO: 17 - DNA, 120 bp, synthetic construct
  source 1..120: mol_type = other DNA
gaggtcagggatggtccagacagaagcacagtaccgatttatctatatggcggtccagcattatattgaaacactacagcgcaggattgaagaagagcaggtaccagcctgagggctggc

SEQ ID NO: 18 - DNA, 120 bp, synthetic construct
  source 1..120: mol_type = other DNA
taggaaatagcagcctcacattgcccctgacaacatagttggaatcactcatgatatctcgagccaatccaaagtcacatatcttcaccactttcccgtgggtgacaagcacgttcctgg

SEQ ID NO: 19 - DNA, 120 bp, synthetic construct
  source 1..120: mol_type = other DNA
ttgcccctgacaacatagttggaatcactcatgatatctcgagccaatccaaagtcacatatcttcaccactttcccgtgggtgacaagcacgttcctggcggccaggtctctgtgaaca

SEQ ID NO: 20 - DNA, 120 bp, synthetic construct
  source 1..120: mol_type = other DNA
gttacctgacagtgtgcacgcccccagcaggttcacaatattctcgtggcttcccagctgggtcatcatcttgagttctgacatgagtgcctctctttcagagctgtctgctttttctgt

SEQ ID NO: 21 - DNA, 120 bp, synthetic construct
  source 1..120: mol_type = other DNA
cccccagcaggttcacaatattctcgtggcttcccagctgggtcatcatcttgagttctgacatgagtgcctctctttcagagctgtctgctttttctgtcaaagaaaggagcattaaaa

SEQ ID NO: 22 - DNA, 120 bp, synthetic construct
  source 1..120: mol_type = other DNA
cattccattcttaccaaactctaaattttctcttggaaactcccatttgagatcatattcatattctctgaaatcaacgtagaagtactcattatctgaggagccggtcacctgtaccat

SEQ ID NO: 23 - DNA, 120 bp, synthetic construct
  source 1..120: mol_type = other DNA
ctaaattttctcttggaaactcccatttgagatcatattcatattctctgaaatcaacgtagaagtactcattatctgaggagccggtcacctgtaccatctgtagctggctttcatacc

SEQ ID NO: 24 - DNA, 120 bp, synthetic construct
  source 1..120: mol_type = other DNA
tattacttgggagacttgtctgaacacttcttccaggtccaagatggtaatgggtatccatccgagaaacaggacgcctgacttgccgatgcttctgcgagcacttgaggtttccctata

SEQ ID NO: 25 - DNA, 120 bp, synthetic construct
  source 1..120: mol_type = other DNA
tgaacacttcttccaggtccaagatggtaatgggtatccatccgagaaacaggacgcctgacttgccgatgcttctgcgagcacttgaggtttccctatagaaaagaacgtgtgaaataa

SEQ ID NO: 26 - DNA, 120 bp, synthetic construct
  source 1..120: mol_type = other DNA
ccctctccaccctggcctacctggtcgccatgggcgtgcctgccaatggtgatgggcttggtccagccagggactaggcgtgggatgtttttgcagatgatgggctcccggaagacagtc

SEQ ID NO: 27 - DNA, 120 bp, synthetic construct
  source 1..120: mol_type = other DNA
tgccaatggtgatgggcttggtccagccagggactaggcgtgggatgtttttgcagatgatgggctcccggaagacagtcccccccaggatgttccggatagttccattgggacttttcc

SEQ ID NO: 28 - DNA, 120 bp, synthetic construct
  source 1..120: mol_type = other DNA
cactcacctggagtgagccctgctcccccctggctccttcccagcctgggcatccttgagttccaaggcctcattcagctctcggaacatctcgaagcgctcacgcccacggatctgcag

SEQ ID NO: 29 - DNA, 120 bp, synthetic construct
  source 1..120: mol_type = other DNA
tgctcccccctggctccttcccagcctgggcatccttgagttccaaggcctcattcagctctcggaacatctcgaagcgctcacgcccacggatctgcagcaacagaggagggggagaag

SEQ ID NO: 30 - DNA, 120 bp, synthetic construct
  source 1..120: mol_type = other DNA
gtgctccctgggggcagctcgtggtgaggctcccctttcttgcggagattctcttcctctgtgcgccggtctctcccaggacaggcacaaacacgcacctcaaagctgttccgtcccagt

SEQ ID NO: 31 - DNA, 120 bp, synthetic construct
  source 1..120: mol_type = other DNA
gtggtgaggctcccctttcttgcggagattctcttcctctgtgcgccggtctctcccaggacaggcacaaacacgcacctcaaagctgttccgtcccagtagattaccactactcaggat

SEQ ID NO: 32 - DNA, 120 bp, synthetic construct
  source 1..120: mol_type = other DNA
ctgacctggagtcttccagtgtgatgatggtgaggatgggcctccggttcatgccgcccatgcaggaactgttacacatgtagttgtagtggatggtggtacagtcagagccaacctagg

SEQ ID NO: 33 - DNA, 120 bp, synthetic construct
  source 1..120: mol_type = other DNA
gtgatgatggtgaggatgggcctccggttcatgccgcccatgcaggaactgttacacatgtagttgtagtggatggtggtacagtcagagccaacctaggagataacacaggcccaagat

SEQ ID NO: 34 - DNA, 120 bp, synthetic construct
  source 1..120: mol_type = other DNA
agacctcaggcggctcatagggcaccaccacactatgtcgaaaagtgtttctgtcatccaaatactccacacgcaaatttccttccactcggataagatgctgaggaggggccagaccta

SEQ ID NO: 35 - DNA, 120 bp, synthetic construct
  source 1..120: mol_type = other DNA
ggcaccaccacactatgtcgaaaagtgtttctgtcatccaaatactccacacgcaaatttccttccactcggataagatgctgaggaggggccagacctaagagcaatcagtgaggaatc

SEQ ID NO: 36 - DNA, 120 bp, synthetic construct
  source 1..120: mol_type = other DNA
ctccagccccagctgctcaccatcgctatctgagcagcgctcatggtgggggcagcgcctcacaacctccgtcatgtgctgtgactgcttgtagatggccatggcgcggacgcgggtgcc

SEQ ID NO: 37 - DNA, 120 bp, synthetic construct
  source 1..120: mol_type = other DNA
gcctcacaacctccgtcatgtgctgtgactgcttgtagatggccatggcgcggacgcgggtgccgggcgggggtgtggaatcaacccacagctgcacagggcaggtcttggccagttggc

SEQ ID NO: 38 - DNA, 120 bp, synthetic construct
  source 1..120: mol_type = other DNA
cgcggacgcgggtgccgggcgggggtgtggaatcaacccacagctgcacagggcaggtcttggccagttggcaaaacatcttgttgagggcaggggagtactgtaggaagaggaaggaga

SEQ ID NO: 39 - DNA, 120 bp, synthetic construct
  source 1..120: mol_type = other DNA
aatgcaagaagcccagacggaaaccgtagctgccctggtaggttttctgggaagggacagaagatgacaggggccaggagggggctggtgcaggggccgccggtgtaggagctgctggtg

SEQ ID NO: 40 - DNA, 120 bp, synthetic construct
  source 1..120: mol_type = other DNA
gaagggacagaagatgacaggggccaggagggggctggtgcaggggccgccggtgtaggagctgctggtgcaggggccacggggggagcagcctctggcattctgggagcttcatctgga

SEQ ID NO: 41 - DNA, 120 bp, synthetic construct
  source 1..120: mol_type = other DNA
gcccttccaatggatccactcacagtttccataggtctgaaaatgtttcctgactcagagggggctcgacgctaggatctgactgcggctcctccatggcagtgacccggaaggcagtct

SEQ ID NO: 42 - DNA, 120 bp, synthetic construct
  source 1..120: mol_type = other DNA
cacagtttccataggtctgaaaatgtttcctgactcagagggggctcgacgctaggatctgactgcggctcctccatggcagtgacccggaaggcagtctggctgctgcaagaggaaaag

SEQ ID NO: 43 - DNA, 120 bp, synthetic construct
  source 1..120: mol_type = other DNA
ttattgccaacatgacttacttgatccccataagcatgacgacctatgatgataggttttacccatccactcacaagccgggggatatttttgcagataatggcttctctgaagaccgtg

SEQ ID NO: 44 - DNA, 120 bp, synthetic construct
  source 1..120: mol_type = other DNA
aggttttacccatccactcacaagccgggggatatttttgcagataatggcttctctgaagaccgtgccacccagaatatttcgtatggtgccatttggtgatttccacatttgtttcaa

SEQ ID NO: 45 - DNA, 35 bp, synthetic construct
  source 1..35: mol_type = other DNA
caaatgctgaaagctgtaccatacctgtctggtct

SEQ ID NO: 46 - DNA, 35 bp, synthetic construct
  source 1..35: mol_type = other DNA
gctgaggtttcaatgaatggaatcccgtaactctt

SEQ ID NO: 47 - DNA, 35 bp, synthetic construct
  source 1..35: mol_type = other DNA
ccagttcgtgggcttgttttgtatcaactgtcctt

SEQ ID NO: 48 - DNA, 35 bp, synthetic construct
  source 1..35: mol_type = other DNA
tggcaaatcacacttgtttcccactagcaccatag

SEQ ID NO: 49 - DNA, 35 bp, synthetic construct
  source 1..35: mol_type = other DNA
acatcatccgagtcttttactcgcttaatctgctc

SEQ ID NO: 50 - DNA, 37 bp, synthetic construct
  source 1..37: mol_type = other DNA
acttgctattattgatggcaaatacacagaggaagcc

SEQ ID NO: 51 - DNA, 35 bp, synthetic construct
  source 1..35: mol_type = other DNA
cgcctgtcctcatgtattggtctctcatggcactg

SEQ ID NO: 52 - DNA, 35 bp, synthetic construct
  source 1..35: mol_type = other DNA
ctcttcttgtccagctgtatccagtatgtccaaca

SEQ ID NO: 53 - DNA, 40 bp, synthetic construct
  source 1..40: mol_type = other DNA
caggtttcaccatctataaccacttgttttctgtaagaat

SEQ ID NO: 54 - DNA, 35 bp, synthetic construct
  source 1..35: mol_type = other DNA
cctgggggtgtggagggtaagggggcagggaggga

SEQ ID NO: 55 - DNA, 35 bp, synthetic construct
  source 1..35: mol_type = other DNA
gggctaccactgggcctcacctctatggtgggatc

SEQ ID NO: 56 - DNA, 38 bp, synthetic construct
  source 1..38: mol_type = other DNA
attcatctacaaagtggttctggattagctggattgtc

SEQ ID NO: 57 - DNA, 35 bp, synthetic construct
  source 1..35: mol_type = other DNA
tgcgcttttcccaacaccacctgctccaaccacca

SEQ ID NO: 58 - DNA, 35 bp, synthetic construct
  source 1..35: mol_type = other DNA
agtttgtactcagtcatttcacaccagcaagaacc

SEQ ID NO: 59 - DNA, 40 bp, synthetic construct
  source 1..40: mol_type = other DNA
tatttatttcagtgttacttacctgtcttgtctttgctga

SEQ ID NO: 60 - DNA, 40 bp, synthetic construct
  source 1..40: mol_type = other DNA
tgtttcaataaaaggaattccataacttcttgctaagtcc

SEQ ID NO: 61 - DNA, 35 bp, synthetic construct
  source 1..35: mol_type = other DNA
tgagcctgttttgtgtctactgttctagaaggcaa

SEQ ID NO: 62 - DNA, 39 bp, synthetic construct
  source 1..39: mol_type = other DNA
cacatttatttcctactaggaccataggtacatcttcag

SEQ ID NO: 63 - DNA, 40 bp, synthetic construct
  source 1..40: mol_type = other DNA
gtccttaactcttttaatttgttctctgggaaagaaaaaa

SEQ ID NO: 64 - DNA, 40 bp, synthetic construct
  source 1..40: mol_type = other DNA
aagttatagcacagtcattagtaacacaaatatctttcaa

SEQ ID NO: 65 - DNA, 40 bp, synthetic construct
  source 1..40: mol_type = other DNA
tagtattatttatggcaaatacacaaagaaagccctcccc

SEQ ID NO: 66 - DNA, 35 bp, synthetic construct
  source 1..35: mol_type = other DNA
agtcctcatgtactggtccctcattgcactgtact

SEQ ID NO: 67 - DNA, 35 bp, synthetic construct
  source 1..35: mol_type = other DNA
tcttgacctgctgtgtcgagaatatccaagagaca

SEQ ID NO: 68 - DNA, 38 bp, synthetic construct
  source 1..38: mol_type = other DNA
tttctccatcaattactacttgcttcctgtaggaatcc

SEQ ID NO: 69 - DNA, 35 bp, synthetic construct
  source 1..35: mol_type = other DNA
agaagggagaaacacagtctggattattacagtgc

SEQ ID NO: 70 - DNA, 40 bp, synthetic construct
  source 1..40: mol_type = other DNA
gatttacctctattgttggatcatattcgtccacaaaatg

SEQ ID NO: 71 - DNA, 35 bp, synthetic construct
  source 1..35: mol_type = other DNA
attctgaattagctgtatcgtcaaggcactcttgc

SEQ ID NO: 72 - DNA, 35 bp, synthetic construct
  source 1..35: mol_type = other DNA
acgccaccagctccaactaccacaagtttatattc

SEQ ID NO: 73 - DNA, 40 bp, synthetic construct
  source 1..40: mol_type = other DNA
tcattttcagcaggccttataataaaaataatgaaaatgt

SEQ ID NO: 74 - DNA, 39 bp, synthetic construct
  source 1..39: mol_type = other DNA
ctttccaatggactattttagaagaaatggagctgtcac

SEQ ID NO: 75 - DNA, 37 bp, synthetic construct
  source 1..37: mol_type = other DNA
cacatcaagattcagaacactggtgattactatgacc

SEQ ID NO: 76 - DNA, 35 bp, synthetic construct
  source 1..35: mol_type = other DNA
tatggaggggagaaatttgccactttggctgagtt

SEQ ID NO: 77 - DNA, 38 bp, synthetic construct
  source 1..38: mol_type = other DNA
tccagtattacatggaacatcacgggcaattaaaagag

SEQ ID NO: 78 - DNA, 39 bp, synthetic construct
  source 1..39: mol_type = other DNA
gaatggagatgtcattgagcttaaatatcctctgaactg

SEQ ID NO: 79 - DNA, 35 bp, synthetic construct
  source 1..35: mol_type = other DNA
cttcatgatgtttccttcgtaggtgttgactgcga

SEQ ID NO: 80 - DNA, 35 bp, synthetic construct
  source 1..35: mol_type = other DNA
ttgacgttcccaaaaccatccagatggtgcggtct

SEQ ID NO: 81 - DNA, 38 bp, synthetic construct
  source 1..38: mol_type = other DNA
gtaccgatttatctatatggcggtccagcattatattg

SEQ ID NO: 82 - DNA, 35 bp, synthetic construct
  source 1..35: mol_type = other DNA
acactacagcgcaggattgaagaagagcaggtacc

SEQ ID NO: 83 - DNA, 35 bp, synthetic construct
  source 1..35: mol_type = other DNA
cctgagggctggcatgcggattctcattctcttgc

SEQ ID NO: 84 - DNA, 35 bp, synthetic construct
  source 1..35: mol_type = other DNA
taagtaggaaatagcagcctcacattgcccctgac

SEQ ID NO: 85 - DNA, 36 bp, synthetic construct
  source 1..36: mol_type = other DNA
catagttggaatcactcatgatatctcgagccaatc

SEQ ID NO: 86 - DNA, 35 bp, synthetic construct
  source 1..35: mol_type = other DNA
aagtcacatatcttcaccactttcccgtgggtgac

SEQ ID NO: 87 - DNA, 35 bp, synthetic construct
  source 1..35: mol_type = other DNA
gcacgttcctggcggccaggtctctgtgaacacac

SEQ ID NO: 88 - DNA, 35 bp, synthetic construct
  source 1..35: mol_type = other DNA
gtgggttacctgacagtgtgcacgcccccagcagg

SEQ ID NO: 89 - DNA, 35 bp, synthetic construct
  source 1..35: mol_type = other DNA
cacaatattctcgtggcttcccagctgggtcatca

SEQ ID NO: 90 - DNA, 35 bp, synthetic construct
  source 1..35: mol_type = other DNA
ttgagttctgacatgagtgcctctctttcagagct

SEQ ID NO: 91 - DNA, 40 bp, synthetic construct
  source 1..40: mol_type = other DNA
ctgctttttctgtcaaagaaaggagcattaaaaatgtaaa

SEQ ID NO: 92 - DNA, 40 bp, synthetic construct
  source 1..40: mol_type = other DNA
ggcacattccattcttaccaaactctaaattttctcttgg

SEQ ID NO: 93 - DNA, 40 bp, synthetic construct
  source 1..40: mol_type = other DNA
aaactcccatttgagatcatattcatattctctgaaatca

SEQ ID NO: 94 - DNA, 35 bp, synthetic construct
  source 1..35: mol_type = other DNA
acgtagaagtactcattatctgaggagccggtcac

SEQ ID NO: 95 - DNA, 35 bp, synthetic construct
  source 1..35: mol_type = other DNA
gtaccatctgtagctggctttcatacctaaattgc

SEQ ID NO: 96 - DNA, 36 bp, synthetic construct
  source 1..36: mol_type = other DNA
tattacttgggagacttgtctgaacacttcttccag

SEQ ID NO: 97 - DNA, 35 bp, synthetic construct
  source 1..35: mol_type = other DNA
ccaagatggtaatgggtatccatccgagaaacagg

SEQ ID NO: 98 - DNA, 35 bp, synthetic construct
  source 1..35: mol_type = other DNA
gcctgacttgccgatgcttctgcgagcacttgagg

SEQ ID NO: 99 - DNA, 37 bp, synthetic construct
  source 1..37: mol_type = other DNA
tccctatagaaaagaacgtgtgaaataagctcactgg

SEQ ID NO: 100 - DNA, 35 bp, synthetic construct
  source 1..35: mol_type = other DNA
atcccctctccaccctggcctacctggtcgccatg

SEQ ID NO: 101 - DNA, 35 bp, synthetic construct
  source 1..35: mol_type = other DNA
cgtgcctgccaatggtgatgggcttggtccagcca

SEQ ID NO: 102 - DNA, 35 bp, synthetic construct
  source 1..35: mol_type = other DNA
gactaggcgtgggatgtttttgcagatgatgggct

SEQ ID NO: 103 - DNA, 35 bp, synthetic construct
  source 1..35: mol_type = other DNA
cggaagacagtcccccccaggatgttccggatagt

SEQ ID NO: 104 - DNA, 35 bp, synthetic construct
  source 1..35: mol_type = other DNA
cattgggacttttccacatcttcttcagcttgaac

SEQ ID NO: 105 - DNA, 35 bp, synthetic construct
  source 1..35: mol_type = other DNA
aggtcactcacctggagtgagccctgctcccccct

SEQ ID NO: 106 - DNA, 35 bp, synthetic construct
  source 1..35: mol_type = other DNA
ctccttcccagcctgggcatccttgagttccaagg

SEQ ID NO: 107 - DNA, 35 bp, synthetic construct
  source 1..35: mol_type = other DNA
tcattcagctctcggaacatctcgaagcgctcacg

SEQ ID NO: 108 - DNA, 35 bp, synthetic construct
  source 1..35: mol_type = other DNA
cacggatctgcagcaacagaggagggggagaagta

SEQ ID NO: 109 - DNA, 35 bp, synthetic construct
  source 1..35: mol_type = other DNA
agtgctccctgggggcagctcgtggtgaggctccc

SEQ ID NO: 110 - DNA, 35 bp, synthetic construct
  source 1..35: mol_type = other DNA
ttcttgcggagattctcttcctctgtgcgccggtc

SEQ ID NO: 111 - DNA, 35 bp, synthetic construct
  source 1..35: mol_type = other DNA
tcccaggacaggcacaaacacgcacctcaaagctg

SEQ ID NO: 112 - DNA, 35 bp, synthetic construct
  source 1..35: mol_type = other DNA
ccgtcccagtagattaccactactcaggataggaa

SEQ ID NO: 113 - DNA, 35 bp, synthetic construct
  source 1..35: mol_type = other DNA
ctcctgacctggagtcttccagtgtgatgatggtg

SEQ ID NO: 114 - DNA, 35 bp, synthetic construct
  source 1..35: mol_type = other DNA
gatgggcctccggttcatgccgcccatgcaggaac

SEQ ID NO: 115 - DNA, 35 bp, synthetic construct
  source 1..35: mol_type = other DNA
ttacacatgtagttgtagtggatggtggtacagtc

SEQ ID NO: 116 - DNA, 35 bp, synthetic construct
  source 1..35: mol_type = other DNA
agccaacctaggagataacacaggcccaagatgag

SEQ ID NO: 117 - DNA, 35 bp, synthetic construct
  source 1..35: mol_type = other DNA
ccagacctcaggcggctcatagggcaccaccacac

SEQ ID NO: 118 - DNA, 37 bp, synthetic construct
  source 1..37: mol_type = other DNA
tgtcgaaaagtgtttctgtcatccaaatactccacac

SEQ ID NO: 119 - DNA, 35 bp, synthetic construct
  source 1..35: mol_type = other DNA
aaatttccttccactcggataagatgctgaggagg

SEQ ID NO: 120 - DNA, 35 bp, synthetic construct
  source 1..35: mol_type = other DNA
ccagacctaagagcaatcagtgaggaatcagaggc

SEQ ID NO: 121 - DNA, 35 bp, synthetic construct
  source 1..35: mol_type = other DNA
ctccagccccagctgctcaccatcgctatctgagc

SEQ ID NO: 122 - DNA, 35 bp, synthetic construct
  source 1..35: mol_type = other DNA
cgctcatggtgggggcagcgcctcacaacctccgt

SEQ ID NO: 123 - DNA, 35 bp, synthetic construct
  source 1..35: mol_type = other DNA
tgtgctgtgactgcttgtagatggccatggcgcgg

SEQ ID NO: 124 - DNA, 35 bp, synthetic construct
  source 1..35: mol_type = other DNA
gcgggtgccgggcgggggtgtggaatcaacccaca

SEQ ID NO: 125 - DNA, 35 bp, synthetic construct
  source 1..35: mol_type = other DNA
tgcacagggcaggtcttggccagttggcaaaacat

SEQ ID NO: 126 - DNA, 35 bp, synthetic construct
  source 1..35: mol_type = other DNA
tgttgagggcaggggagtactgtaggaagaggaag

SEQ ID NO: 127 - DNA, 35 bp, synthetic construct
  source 1..35: mol_type = other DNA
gacagagttgaaagtcagggcacaagtgaacagat

SEQ ID NO: 128 - DNA, 35 bp, synthetic construct
  source 1..35: mol_type = other DNA
aatgcaagaagcccagacggaaaccgtagctgccc

SEQ ID NO: 129 - DNA, 35 bp, synthetic construct
  source 1..35: mol_type = other DNA
gtaggttttctgggaagggacagaagatgacaggg

SEQ ID NO: 130 - DNA, 35 bp, synthetic construct
  source 1..35: mol_type = other DNA
caggagggggctggtgcaggggccgccggtgtagg

SEQ ID NO: 131 - DNA, 35 bp, synthetic construct
  source 1..35: mol_type = other DNA
ctgctggtgcaggggccacggggggagcagcctct

SEQ ID NO: 132 - DNA, 35 bp, synthetic construct
  source 1..35: mol_type = other DNA
cattctgggagcttcatctggacctgggtcttcag

SEQ ID NO: 133 - DNA, 35 bp, synthetic construct
  source 1..35: mol_type = other DNA
gcccttccaatggatccactcacagtttccatagg

SEQ ID NO: 134 - DNA, 35 bp, synthetic construct
  source 1..35: mol_type = other DNA
tgaaaatgtttcctgactcagagggggctcgacgc

SEQ ID NO: 135 - DNA, 35 bp, synthetic construct
  source 1..35: mol_type = other DNA
ggatctgactgcggctcctccatggcagtgacccg

SEQ ID NO: 136 - DNA, 35 bp, synthetic construct
  source 1..35: mol_type = other DNA
aggcagtctggctgctgcaagaggaaaagtgggga

SEQ ID NO: 137 - DNA, 37 bp, synthetic construct
  source 1..37: mol_type = other DNA
cattattgccaacatgacttacttgatccccataagc

SEQ ID NO: 138 - DNA, 35 bp, synthetic construct
  source 1..35: mol_type = other DNA
gacgacctatgatgataggttttacccatccactc

SEQ ID NO: 139 - DNA, 35 bp, synthetic construct
  source 1..35: mol_type = other DNA
aagccgggggatatttttgcagataatggcttctc

SEQ ID NO: 140 - DNA, 35 bp, synthetic construct
  source 1..35: mol_type = other DNA
aagaccgtgccacccagaatatttcgtatggtgcc

SEQ ID NO: 141 - DNA, 40 bp, synthetic construct
  source 1..40: mol_type = other DNA
ttggtgatttccacatttgtttcaacttgaactcctcaac

SEQ ID NO: 142 - DNA, 51 bp, synthetic construct
  source 1..51: mol_type = other DNA
cgtcggtccaaatgctgaaagctgtaccatacctgtctggtctgaccgacg

SEQ ID NO: 143 - DNA, 51 bp, synthetic construct
  source 1..51: mol_type = other DNA
cgtcggtcgctgaggtttcaatgaatggaatcccgtaactcttgaccgacg

SEQ ID NO: 144 - DNA, 51 bp, synthetic construct
  source 1..51: mol_type = other DNA
cgtcggtcccagttcgtgggcttgttttgtatcaactgtccttgaccgacg

SEQ ID NO: 145 - DNA, 51 bp, synthetic construct
  source 1..51: mol_type = other DNA
cgtcggtctggcaaatcacacttgtttcccactagcaccataggaccgacg

SEQ ID NO: 146 - DNA, 51 bp, synthetic construct
  source 1..51: mol_type = other DNA
cgtcggtcacatcatccgagtcttttactcgcttaatctgctcgaccgacg

SEQ ID NO: 147 - DNA, 53 bp, synthetic construct
  source 1..53: mol_type = other DNA
cgtcggtcacttgctattattgatggcaaatacacagaggaagccgaccgacg

SEQ ID NO: 148 - DNA, 51 bp, synthetic construct
  source 1..51: mol_type = other DNA
cgtcggtccgcctgtcctcatgtattggtctctcatggcactggaccgacg

SEQ ID NO: 149 - DNA, 51 bp, synthetic construct
  source 1..51: mol_type = other DNA
cgtcggtcctcttcttgtccagctgtatccagtatgtccaacagaccgacg

SEQ ID NO: 150 - DNA, 56 bp, synthetic construct
  source 1..56: mol_type = other DNA
cgtcggtccaggtttcaccatctataaccacttgttttctgtaagaatgaccgacg

SEQ ID NO: 151 - DNA, 51 bp, synthetic construct
  source 1..51: mol_type = other DNA
cgtcggtccctgggggtgtggagggtaagggggcagggagggagaccgacg

SEQ ID NO: 152 - DNA, 51 bp, synthetic construct
  source 1..51: mol_type = other DNA
cgtcggtcgggctaccactgggcctcacctctatggtgggatcgaccgacg

SEQ ID NO: 153 - DNA, 54 bp, synthetic construct
  source 1..54: mol_type = other DNA
cgtcggtcattcatctacaaagtggttctggattagctggattgtcgaccgacg

SEQ ID NO: 154 - DNA, 51 bp, synthetic construct
  source 1..51: mol_type = other DNA
cgtcggtctgcgcttttcccaacaccacctgctccaaccaccagaccgacg

SEQ ID NO: 155 - DNA, 51 bp, synthetic construct
  source 1..51: mol_type = other DNA
cgtcggtcagtttgtactcagtcatttcacaccagcaagaaccgaccgacg

SEQ ID NO: 156 - DNA, 56 bp, synthetic construct
  source 1..56: mol_type = other DNA
cgtcggtctatttatttcagtgttacttacctgtcttgtctttgctgagaccgacg

SEQ ID NO: 157 - DNA, 56 bp, synthetic construct
  source 1..56: mol_type = other DNA
cgtcggtctgtttcaataaaaggaattccataacttcttgctaagtccgaccgacg

SEQ ID NO: 158 - DNA, 51 bp, synthetic construct
  source 1..51: mol_type = other DNA
cgtcggtctgagcctgttttgtgtctactgttctagaaggcaagaccgacg

SEQ ID NO: 159 - DNA, 55 bp, synthetic construct
  source 1..55: mol_type = other DNA
cgtcggtccacatttatttcctactaggaccataggtacatcttcaggaccgacg

SEQ ID NO: 160 - DNA, 56 bp, synthetic construct
  source 1..56: mol_type = other DNA
cgtcggtcgtccttaactcttttaatttgttctctgggaaagaaaaaagaccgacg

SEQ ID NO: 161 - DNA, 56 bp, synthetic construct
  source 1..56: mol_type = other DNA
cgtcggtcaagttatagcacagtcattagtaacacaaatatctttcaagaccgacg

SEQ ID NO: 162 - DNA, 56 bp, synthetic construct
  source 1..56: mol_type = other DNA
cgtcggtctagtattatttatggcaaatacacaaagaaagccctccccgaccgacg

SEQ ID NO: 163 - DNA, 51 bp, synthetic construct
  source 1..51: mol_type = other DNA
cgtcggtcagtcctcatgtactggtccctcattgcactgtactgaccgacg

SEQ ID NO: 164 - DNA, 51 bp, synthetic construct
  source 1..51: mol_type = other DNA
cgtcggtctcttgacctgctgtgtcgagaatatccaagagacagaccgacg

SEQ ID NO: 165 - DNA, 54 bp, synthetic construct
  source 1..54: mol_type = other DNA
cgtcggtctttctccatcaattactacttgcttcctgtaggaatccgaccgacg

SEQ ID NO: 166 - DNA, 51 bp, synthetic construct
  source 1..51: mol_type = other DNA
cgtcggtcagaagggagaaacacagtctggattattacagtgcgaccgacg

SEQ ID NO: 167 - DNA, 56 bp, synthetic construct
  source 1..56: mol_type = other DNA
cgtcggtcgatttacctctattgttggatcatattcgtccacaaaatggaccgacg

SEQ ID NO: 168 - DNA, 51 bp, synthetic construct
  source 1..51: mol_type = other DNA
cgtcggtcattctgaattagctgtatcgtcaaggcactcttgcgaccgacg

SEQ ID NO: 169 - DNA, 51 bp, synthetic construct
  source 1..51: mol_type = other DNA
cgtcggtcacgccaccagctccaactaccacaagtttatattcgaccgacg

SEQ ID NO: 170 - DNA, 56 bp, synthetic construct
  source 1..56: mol_type = other DNA
cgtcggtctcattttcagcaggccttataataaaaataatgaaaatgtgaccgacg

SEQ ID NO: 171 - DNA, 55 bp, synthetic construct
  source 1..55: mol_type = other DNA
cgtcggtcctttccaatggactattttagaagaaatggagctgtcacgaccgacg

SEQ ID NO: 172 - DNA, 53 bp, synthetic construct
  source 1..53: mol_type = other DNA
cgtcggtccacatcaagattcagaacactggtgattactatgaccgaccgacg

SEQ ID NO: 173 - DNA, 51 bp, synthetic construct
  source 1..51: mol_type = other DNA
cgtcggtctatggaggggagaaatttgccactttggctgagttgaccgacg

SEQ ID NO: 174 - DNA, 54 bp, synthetic construct
  source 1..54: mol_type = other DNA
cgtcggtctccagtattacatggaacatcacgggcaattaaaagaggaccgacg

SEQ ID NO: 175 - DNA, 55 bp, synthetic construct
  source 1..55: mol_type = other DNA
cgtcggtcgaatggagatgtcattgagcttaaatatcctctgaactggaccgacg

SEQ ID NO: 176 - DNA, 51 bp, synthetic construct
  source 1..51: mol_type = other DNA
cgtcggtccttcatgatgtttccttcgtaggtgttgactgcgagaccgacg

SEQ ID NO: 177 - DNA, 51 bp, synthetic construct
  source 1..51: mol_type = other DNA
cgtcggtcttgacgttcccaaaaccatccagatggtgcggtctgaccgacg

SEQ ID NO: 178 - DNA, 54 bp, synthetic construct
  source 1..54: mol_type = other DNA
cgtcggtcgtaccgatttatctatatggcggtccagcattatattggaccgacg

SEQ ID NO: 179 - DNA, 51 bp, synthetic construct
  source 1..51: mol_type = other DNA
cgtcggtcacactacagcgcaggattgaagaagagcaggtaccgaccgacg

SEQ ID NO: 180 - DNA, 51 bp, synthetic construct
  source 1..51: mol_type = other DNA
cgtcggtccctgagggctggcatgcggattctcattctcttgcgaccgacg

SEQ ID NO: 181 - DNA, 51 bp, synthetic construct
  source 1..51: mol_type = other DNA
cgtcggtctaagtaggaaatagcagcctcacattgcccctgacgaccgacg

SEQ ID NO: 182 - DNA, 52 bp, synthetic construct
  source 1..52: mol_type = other DNA
cgtcggtccatagttggaatcactcatgatatctcgagccaatcgaccgacg

SEQ ID NO: 183 - DNA, 51 bp, synthetic construct
  source 1..51: mol_type = other DNA
cgtcggtcaagtcacatatcttcaccactttcccgtgggtgacgaccgacg

SEQ ID NO: 184 - DNA, 51 bp, synthetic construct
  source 1..51: mol_type = other DNA
cgtcggtcgcacgttcctggcggccaggtctctgtgaacacacgaccgacg

SEQ ID NO: 185 - DNA, 51 bp, synthetic construct
  source 1..51: mol_type = other DNA
cgtcggtcgtgggttacctgacagtgtgcacgcccccagcagggaccgacg

SEQ ID NO: 186 - DNA, 51 bp, synthetic construct
  source 1..51: mol_type = other DNA
cgtcggtccacaatattctcgtggcttcccagctgggtcatcagaccgacg

SEQ ID NO: 187 - DNA, 51 bp, synthetic construct
  source 1..51: mol_type = other DNA
cgtcggtcttgagttctgacatgagtgcctctctttcagagctgaccgacg

SEQ ID NO: 188 - DNA, 56 bp, synthetic construct
  source 1..56: mol_type = other DNA
cgtcggtcctgctttttctgtcaaagaaaggagcattaaaaatgtaaagaccgacg

SEQ ID NO: 189 - DNA, 56 bp, synthetic construct
  source 1..56: mol_type = other DNA
cgtcggtcggcacattccattcttaccaaactctaaattttctcttgggaccgacg

SEQ ID NO: 190 - DNA, 56 bp, synthetic construct
  source 1..56: mol_type = other DNA
cgtcggtcaaactcccatttgagatcatattcatattctctgaaatcagaccgacg

SEQ ID NO: 191 - DNA, 51 bp, synthetic construct
  source 1..51: mol_type = other DNA
cgtcggtcacgtagaagtactcattatctgaggagccggtcacgaccgacg

SEQ ID NO: 192 - DNA, 51 bp, synthetic construct
  source 1..51: mol_type = other DNA
cgtcggtcgtaccatctgtagctggctttcatacctaaattgcgaccgacg

SEQ ID NO: 193 - DNA, 52 bp, synthetic construct
  source 1..52: mol_type = other DNA
cgtcggtctattacttgggagacttgtctgaacacttcttccaggaccgacg

SEQ ID NO: 194 - DNA, 51 bp, synthetic construct
  source 1..51: mol_type = other DNA
cgtcggtcccaagatggtaatgggtatccatccgagaaacagggaccgacg

SEQ ID NO: 195 - DNA, 51 bp, synthetic construct
  source 1..51: mol_type = other DNA
cgtcggtcgcctgacttgccgatgcttctgcgagcacttgagggaccgacg

SEQ ID NO: 196 - DNA, 53 bp, synthetic construct
  source 1..53: mol_type = other DNA
cgtcggtctccctatagaaaagaacgtgtgaaataagctcactgggaccgacg

SEQ ID NO: 197 - DNA, 51 bp, synthetic construct
  source 1..51: mol_type = other DNA
cgtcggtcatcccctctccaccctggcctacctggtcgccatggaccgacg

SEQ ID NO: 198 - DNA, 51 bp, synthetic construct
  source 1..51: mol_type = other DNA
cgtcggtccgtgcctgccaatggtgatgggcttggtccagccagaccgacg

SEQ ID NO: 199 - DNA, 51 bp, synthetic construct
  source 1..51: mol_type = other DNA
cgtcggtcgactaggcgtgggatgtttttgcagatgatgggctgaccgacg

SEQ ID NO: 200 - DNA, 51 bp, synthetic construct
  source 1..51: mol_type = other DNA
cgtcggtccggaagacagtcccccccaggatgttccggatagtgaccgacg

SEQ ID NO: 201 - DNA, 51 bp, synthetic construct
  source 1..51: mol_type = other DNA
cgtcggtccattgggacttttccacatcttcttcagcttgaacgaccgacg

SEQ ID NO: 202 - DNA, 51 bp, synthetic construct
  source 1..51: mol_type = other DNA
cgtcggtcaggtcactcacctggagtgagccctgctcccccctgaccgacg

SEQ ID NO: 203 - DNA, 51 bp, synthetic construct
  source 1..51: mol_type = other DNA
cgtcggtcctccttcccagcctgggcatccttgagttccaagggaccgacg

SEQ ID NO: 204 - DNA, 51 bp, synthetic construct
  source 1..51: mol_type = other DNA
cgtcggtctcattcagctctcggaacatctcgaagcgctcacggaccgacg

SEQ ID NO: 205 - DNA, 51 bp, synthetic construct
  source 1..51: mol_type = other DNA
cgtcggtccacggatctgcagcaacagaggagggggagaagtagaccgacg

SEQ ID NO: 206 - DNA, 51 bp, synthetic construct
  source 1..51: mol_type = other DNA
cgtcggtcagtgctccctgggggcagctcgtggtgaggctcccgaccgacg

SEQ ID NO: 207 - DNA, 51 bp, synthetic construct
  source 1..51: mol_type = other DNA
cgtcggtcttcttgcggagattctcttcctctgtgcgccggtcgaccgacg

SEQ ID NO: 208 - DNA, 51 bp, synthetic construct
  source 1..51: mol_type = other DNA
cgtcggtctcccaggacaggcacaaacacgcacctcaaagctggaccgacg

SEQ ID NO: 209 - DNA, 51 bp, synthetic construct
  source 1..51: mol_type = other DNA
cgtcggtcccgtcccagtagattaccactactcaggataggaagaccgacg

SEQ ID NO: 210 - DNA, 51 bp, synthetic construct
  source 1..51: mol_type = other DNA
cgtcggtcctcctgacctggagtcttccagtgtgatgatggtggaccgacg

SEQ ID NO: 211 - DNA, 51 bp, synthetic construct
  source 1..51: mol_type = other DNA
cgtcggtcgatgggcctccggttcatgccgcccatgcaggaacgaccgacg

SEQ ID NO: 212 - DNA, 51 bp, synthetic construct
  source 1..51: mol_type = other DNA
cgtcggtcttacacatgtagttgtagtggatggtggtacagtcgaccgacg

SEQ ID NO: 213 - DNA, 51 bp, synthetic construct
  source 1..51: mol_type = other DNA
cgtcggtcagccaacctaggagataacacaggcccaagatgaggaccgacg

SEQ ID NO: 214 - DNA, 51 bp, synthetic construct
  source 1..51: mol_type = other DNA
cgtcggtcccagacctcaggcggctcatagggcaccaccacacgaccgacg

SEQ ID NO: 215 - DNA, 53 bp, synthetic construct
  source 1..53: mol_type = other DNA
cgtcggtctgtcgaaaagtgtttctgtcatccaaatactccacacgaccgacg

SEQ ID NO: 216 - DNA, 51 bp, synthetic construct
  source 1..51: mol_type = other DNA
cgtcggtcaaatttccttccactcggataagatgctgaggagggaccgacg

SEQ ID NO: 217 - DNA, 51 bp, synthetic construct
  source 1..51: mol_type = other DNA
cgtcggtcccagacctaagagcaatcagtgaggaatcagaggcgaccgacg

SEQ ID NO: 218 - DNA, 51 bp, synthetic construct
  source 1..51: mol_type = other DNA
cgtcggtcctccagccccagctgctcaccatcgctatctgagcgaccgacg

SEQ ID NO: 219 - DNA, 51 bp, synthetic construct
  source 1..51: mol_type = other DNA
cgtcggtccgctcatggtgggggcagcgcctcacaacctccgtgaccgacg

SEQ ID NO: 220 - DNA, 51 bp, synthetic construct
  source 1..51: mol_type = other DNA
cgtcggtctgtgctgtgactgcttgtagatggccatggcgcgggaccgacg

SEQ ID NO: 221 - DNA, 51 bp, synthetic construct
  source 1..51: mol_type = other DNA
cgtcggtcgcgggtgccgggcgggggtgtggaatcaacccacagaccgacg

SEQ ID NO: 222 - DNA, 51 bp, synthetic construct
  source 1..51: mol_type = other DNA
cgtcggtctgcacagggcaggtcttggccagttggcaaaacatgaccgacg

SEQ ID NO: 223 - DNA, 51 bp, synthetic construct
  source 1..51: mol_type = other DNA
cgtcggtctgttgagggcaggggagtactgtaggaagaggaaggaccgacg

SEQ ID NO: 224 - DNA, 51 bp, synthetic construct
  source 1..51: mol_type = other DNA
cgtcggtcgacagagttgaaagtcagggcacaagtgaacagatgaccgacg

SEQ ID NO: 225 - DNA, 51 bp, synthetic construct
  source 1..51: mol_type = other DNA
cgtcggtcaatgcaagaagcccagacggaaaccgtagctgcccgaccgacg

SEQ ID NO: 226 - DNA, 51 bp, synthetic construct
  source 1..51: mol_type = other DNA
cgtcggtcgtaggttttctgggaagggacagaagatgacaggggaccgacg

SEQ ID NO: 227 - DNA, 51 bp, synthetic construct
  source 1..51: mol_type = other DNA
cgtcggtccaggagggggctggtgcaggggccgccggtgtagggaccgacg

SEQ ID NO: 228 - DNA, 51 bp, synthetic construct
  source 1..51: mol_type = other DNA
cgtcggtcctgctggtgcaggggccacggggggagcagcctctgaccgacg

SEQ ID NO: 229 - DNA, 51 bp, synthetic construct
  source 1..51: mol_type = other DNA
cgtcggtccattctgggagcttcatctggacctgggtcttcaggaccgacg

SEQ ID NO: 230 - DNA, 51 bp, synthetic construct
  source 1..51: mol_type = other DNA
cgtcggtcgcccttccaatggatccactcacagtttccatagggaccgacg

SEQ ID NO: 231 - DNA, 51 bp, synthetic construct
  source 1..51: mol_type = other DNA
cgtcggtctgaaaatgtttcctgactcagagggggctcgacgcgaccgacg

SEQ ID NO: 232 - DNA, 51 bp, synthetic construct
  source 1..51: mol_type = other DNA
cgtcggtcggatctgactgcggctcctccatggcagtgacccggaccgacg

SEQ ID NO: 233 - DNA, 51 bp, synthetic construct
  source 1..51: mol_type = other DNA
cgtcggtcaggcagtctggctgctgcaagaggaaaagtggggagaccgacg

SEQ ID NO: 234 - DNA, 53 bp, synthetic construct
  source 1..53: mol_type = other DNA
cgtcggtccattattgccaacatgacttacttgatccccataagcgaccgacg

SEQ ID NO: 235 - DNA, 51 bp, synthetic construct
  source 1..51: mol_type = other DNA
cgtcggtcgacgacctatgatgataggttttacccatccactcgaccgacg

SEQ ID NO: 236 - DNA, 51 bp, synthetic construct
  source 1..51: mol_type = other DNA
cgtcggtcaagccgggggatatttttgcagataatggcttctcgaccgacg

SEQ ID NO: 237 - DNA, 51 bp, synthetic construct
  source 1..51: mol_type = other DNA
cgtcggtcaagaccgtgccacccagaatatttcgtatggtgccgaccgacg

SEQ ID NO: 238 - DNA, 56 bp, synthetic construct
  source 1..56: mol_type = other DNA
cgtcggtcttggtgatttccacatttgtttcaacttgaactcctcaacgaccgacg

SEQ ID NO: 239 - DNA, 120 bp, synthetic construct
  source 1..120: mol_type = other DNA
gtgtgatttgccaacaaggacagttgatacaaaacaagcccacgaactggccaagagttacgggattccattcattgaaacctcagccaagaccagacaggtatggtacagctttcagca

SEQ ID NO: 240 - DNA, 120 bp, synthetic construct
  source 1..120: mol_type = other DNA
aagactcggatgatgtacctatggtgctagtgggaaacaagtgtgatttgccaacaaggacagttgatacaaaacaagcccacgaactggccaagagttacgggattccattcattgaaa

SEQ ID NO: 241 - DNA, 120 bp, synthetic construct
  source 1..120: mol_type = other DNA
ggtgaaacctgtttgttggacatactggatacagctggacaagaagagtacagtgccatgagagaccaatacatgaggacaggcgaaggcttcctctgtgtatttgccatcaataatagc

SEQ ID NO: 242 - DNA, 120 bp, synthetic construct
  source 1..120: mol_type = other DNA
cttaccctccacacccccaggattcttacagaaaacaagtggttatagatggtgaaacctgtttgttggacatactggatacagctggacaagaagagtacagtgccatgagagaccaat

SEQ ID NO: 243 - DNA, 120 bp, synthetic construct
  source 1..120: mol_type = other DNA
agtacaaactggtggtggttggagcaggtggtgttgggaaaagcgcactgacaatccagctaatccagaaccactttgtagatgaatatgatcccaccatagaggtgaggcccagtggta

SEQ ID NO: 244 - DNA, 120 bp, synthetic construct
  source 1..120: mol_type = other DNA
tgaaatgactgagtacaaactggtggtggttggagcaggtggtgttgggaaaagcgcactgacaatccagctaatccagaaccactttgtagatgaatatgatcccaccatagaggtgag

SEQ ID NO: 245 - DNA, 120 bp, synthetic construct
  source 1..120: mol_type = other DNA
atgtgatttgccttctagaacagtagacacaaaacaggctcaggacttagcaagaagttatggaattccttttattgaaacatcagcaaagacaagacaggtaagtaacactgaaataaa

SEQ ID NO: 246 - DNA, 120 bp, synthetic construct
  source 1..120: mol_type = other DNA
aggactctgaagatgtacctatggtcctagtaggaaataaatgtgatttgccttctagaacagtagacacaaaacaggctcaggacttagcaagaagttatggaattccttttattgaaa

SEQ ID NO: 247 - DNA, 120 bp, synthetic construct
  source 1..120: mol_type = other DNA
aacttttttttctttcccagagaacaaattaaaagagttaaggactctgaagatgtacctatggtcctagtaggaaataaatgtgatttgccttctagaacagtagacacaaaacaggct

SEQ ID NO: 248 - DNA, 120 bp, synthetic construct
  source 1..120: mol_type = other DNA
ggagaaacctgtctcttggatattctcgacacagcaggtcaagaggagtacagtgcaatgagggaccagtacatgaggactggggagggctttctttgtgtatttgccataaataatact

SEQ ID NO: 249 - DNA, 120 bp, synthetic construct
  source 1..120: mol_type = other DNA
ctgtgtttctcccttctcaggattcctacaggaagcaagtagtaattgatggagaaacctgtctcttggatattctcgacacagcaggtcaagaggagtacagtgcaatgagggaccagt

SEQ ID NO: 250 - DNA, 120 bp, synthetic construct
  source 1..120: mol_type = other DNA
gaaaatgactgaatataaacttgtggtagttggagctggtggcgtaggcaagagtgccttgacgatacagctaattcagaatcattttgtggacgaatatgatccaacaatagaggtaaa

SEQ ID NO: 251 - DNA, 120 bp, synthetic construct
  source 1..120: mol_type = other DNA
tcattatttttattataaggcctgctgaaaatgactgaatataaacttgtggtagttggagctggtggcgtaggcaagagtgccttgacgatacagctaattcagaatcattttgtggac

SEQ ID NO: 252 - DNA, 120 bp, synthetic construct
  source 1..120: mol_type = other DNA
ctggaccaactcagccaaagtggcaaatttctcccctccatacaggtcatagtaatcaccagtgttctgaatcttgatgtgggtgacagctccatttcttctaaaatagtccattggaaa

SEQ ID NO: 253 - DNA, 120 bp, synthetic construct
  source 1..120: mol_type = other DNA
aagctcaatgacatctccattcttctcttttaattgcccgtgatgttccatgtaatactggaccaactcagccaaagtggcaaatttctcccctccatacaggtcatagtaatcaccagt

SEQ ID NO: 254 - DNA, 120 bp, synthetic construct
  source 1..120: mol_type = other DNA
atatagataaatcggtactgtgcttctgtctggaccatccctgacctctgagaccgcaccatctggatggttttgggaacgtcaatatcgcagtcaacacctacgaaggaaacatcatga

SEQ ID NO: 255 - DNA, 120 bp, synthetic construct
  source 1..120: mol_type = other DNA
gccagccctcaggctggtacctgctcttcttcaatcctgcgctgtagtgtttcaatataatgctggaccgccatatagataaatcggtactgtgcttctgtctggaccatccctgacctc

SEQ ID NO: 256 - DNA, 120 bp, synthetic construct
  source 1..120: mol_type = other DNA
ccaggaacgtgcttgtcacccacgggaaagtggtgaagatatgtgactttggattggctcgagatatcatgagtgattccaactatgttgtcaggggcaatgtgaggctgctatttccta

SEQ ID NO: 257 - DNA, 120 bp, synthetic construct
  source 1..120: mol_type = other DNA
tgttcacagagacctggccgccaggaacgtgcttgtcacccacgggaaagtggtgaagatatgtgactttggattggctcgagatatcatgagtgattccaactatgttgtcaggggcaa

SEQ ID NO: 258 - DNA, 120 bp, synthetic construct
  source 1..120: mol_type = other DNA
acagaaaaagcagacagctctgaaagagaggcactcatgtcagaactcaagatgatgacccagctgggaagccacgagaatattgtgaacctgctgggggcgtgcacactgtcaggtaac

SEQ ID NO: 259 - DNA, 120 bp, synthetic construct
  source 1..120: mol_type = other DNA
ttttaatgctcctttctttgacagaaaaagcagacagctctgaaagagaggcactcatgtcagaactcaagatgatgacccagctgggaagccacgagaatattgtgaacctgctggggg

SEQ ID NO: 260 - DNA, 120 bp, synthetic construct
  source 1..120: mol_type = other DNA
atggtacaggtgaccggctcctcagataatgagtacttctacgttgatttcagagaatatgaatatgatctcaaatgggagtttccaagagaaaatttagagtttggtaagaatggaatg

SEQ ID NO: 261 - DNA, 120 bp, synthetic construct
  source 1..120: mol_type = other DNA
ggtatgaaagccagctacagatggtacaggtgaccggctcctcagataatgagtacttctacgttgatttcagagaatatgaatatgatctcaaatgggagtttccaagagaaaatttag

SEQ ID NO: 262 - DNA, 120 bp, synthetic construct
  source 1..120: mol_type = other DNA
tatagggaaacctcaagtgctcgcagaagcatcggcaagtcaggcgtcctgtttctcggatggatacccattaccatcttggacctggaagaagtgttcagacaagtctcccaagtaata

SEQ ID NO: 263 - DNA, 120 bp, synthetic construct
  source 1..120: mol_type = other DNA
ttatttcacacgttcttttctatagggaaacctcaagtgctcgcagaagcatcggcaagtcaggcgtcctgtttctcggatggatacccattaccatcttggacctggaagaagtgttca

SEQ ID NO: 264 - DNA, 120 bp, synthetic construct
  source 1..120: mol_type = other DNA
gactgtcttccgggagcccatcatctgcaaaaacatcccacgcctagtccctggctggaccaagcccatcaccattggcaggcacgcccatggcgaccaggtaggccagggtggagaggg

SEQ ID NO: 265 - DNA, 120 bp, synthetic construct
  source 1..120: mol_type = other DNA
ggaaaagtcccaatggaactatccggaacatcctgggggggactgtcttccgggagcccatcatctgcaaaaacatcccacgcctagtccctggctggaccaagcccatcaccattggca

SEQ ID NO: 266 - DNA, 120 bp, synthetic construct
  source 1..120: mol_type = other DNA
ctgcagatccgtgggcgtgagcgcttcgagatgttccgagagctgaatgaggccttggaactcaaggatgcccaggctgggaaggagccaggggggagcagggctcactccaggtgagtg

SEQ ID NO: 267 - DNA, 120 bp, synthetic construct
  source 1..120: mol_type = other DNA
cttctccccctcctctgttgctgcagatccgtgggcgtgagcgcttcgagatgttccgagagctgaatgaggccttggaactcaaggatgcccaggctgggaaggagccaggggggagca

SEQ ID NO: 268 - DNA, 120 bp, synthetic construct
  source 1..120: mol_type = other DNA
actgggacggaacagctttgaggtgcgtgtttgtgcctgtcctgggagagaccggcgcacagaggaagagaatctccgcaagaaaggggagcctcaccacgagctgcccccagggagcac

SEQ ID NO: 269 - DNA, 120 bp, synthetic construct
  source 1..120: mol_type = other DNA
atcctgagtagtggtaatctactgggacggaacagctttgaggtgcgtgtttgtgcctgtcctgggagagaccggcgcacagaggaagagaatctccgcaagaaaggggagcctcaccac

SEQ ID NO: 270 - DNA, 120 bp, synthetic construct
  source 1..120: mol_type = other DNA
cctaggttggctctgactgtaccaccatccactacaactacatgtgtaacagttcctgcatgggcggcatgaaccggaggcccatcctcaccatcatcacactggaagactccaggtcag

SEQ ID NO: 271 - DNA, 120 bp, synthetic construct
  source 1..120: mol_type = other DNA
atcttgggcctgtgttatctcctaggttggctctgactgtaccaccatccactacaactacatgtgtaacagttcctgcatgggcggcatgaaccggaggcccatcctcaccatcatcac

SEQ ID NO: 272 - DNA, 120 bp, synthetic construct
  source 1..120: mol_type = other DNA
taggtctggcccctcctcagcatcttatccgagtggaaggaaatttgcgtgtggagtatttggatgacagaaacacttttcgacatagtgtggtggtgccctatgagccgcctgaggtct

SEQ ID NO: 273 - DNA, 120 bp, synthetic construct
  source 1..120: mol_type = other DNA
gattcctcactgattgctcttaggtctggcccctcctcagcatcttatccgagtggaaggaaatttgcgtgtggagtatttggatgacagaaacacttttcgacatagtgtggtggtgcc

SEQ ID NO: 274 - DNA, 120 bp, synthetic construct
  source 1..120: mol_type = other DNA
ggcacccgcgtccgcgccatggccatctacaagcagtcacagcacatgacggaggttgtgaggcgctgcccccaccatgagcgctgctcagatagcgatggtgagcagctggggctggag

SEQ ID NO: 275 - DNA, 120 bp, synthetic construct
  source 1..120: mol_type = other DNA
gccaactggccaagacctgccctgtgcagctgtgggttgattccacacccccgcccggcacccgcgtccgcgccatggccatctacaagcagtcacagcacatgacggaggttgtgaggc

SEQ ID NO: 276 - DNA, 120 bp, synthetic construct
  source 1..120: mol_type = other DNA
tctccttcctcttcctacagtactcccctgccctcaacaagatgttttgccaactggccaagacctgccctgtgcagctgtgggttgattccacacccccgcccggcacccgcgtccgcg

SEQ ID NO: 277 - DNA, 120 bp, synthetic construct
  source 1..120: mol_type = other DNA
caccagcagctcctacaccggcggcccctgcaccagccccctcctggcccctgtcatcttctgtcccttcccagaaaacctaccagggcagctacggtttccgtctgggcttcttgcatt

SEQ ID NO: 278 - DNA, 120 bp, synthetic construct
  source 1..120: mol_type = other DNA
tccagatgaagctcccagaatgccagaggctgctccccccgtggcccctgcaccagcagctcctacaccggcggcccctgcaccagccccctcctggcccctgtcatcttctgtcccttc

SEQ ID NO: 279 - DNA, 120 bp, synthetic construct
  source 1..120: mol_type = other DNA
agactgccttccgggtcactgccatggaggagccgcagtcagatcctagcgtcgagccccctctgagtcaggaaacattttcagacctatggaaactgtgagtggatccattggaagggc

SEQ ID NO: 280 - DNA, 120 bp, synthetic construct
  source 1..120: mol_type = other DNA
cttttcctcttgcagcagccagactgccttccgggtcactgccatggaggagccgcagtcagatcctagcgtcgagccccctctgagtcaggaaacattttcagacctatggaaactgtg

SEQ ID NO: 281 - DNA, 120 bp, synthetic construct
  source 1..120: mol_type = other DNA
cacggtcttcagagaagccattatctgcaaaaatatcccccggcttgtgagtggatgggtaaaacctatcatcataggtcgtcatgcttatggggatcaagtaagtcatgttggcaataa

SEQ ID NO: 282 - DNA, 120 bp, synthetic construct
  source 1..120: mol_type = other DNA
ttgaaacaaatgtggaaatcaccaaatggcaccatacgaaatattctgggtggcacggtcttcagagaagccattatctgcaaaaatatcccccggcttgtgagtggatgggtaaaacct

SEQ ID NO: 283 - DNA, 51 bp, synthetic construct
  source 1..51: mol_type = other DNA
cgtcggtcagaccagacaggtatggtacagctttcagcatttggaccgacg

SEQ ID NO: 284 - DNA, 51 bp, synthetic construct
  source 1..51: mol_type = other DNA
cgtcggtcaagagttacgggattccattcattgaaacctcagcgaccgacg

SEQ ID NO: 285 - DNA, 51 bp, synthetic construct
  source 1..51: mol_type = other DNA
cgtcggtcaaggacagttgatacaaaacaagcccacgaactgggaccgacg

SEQ ID NO: 286 - DNA, 51 bp, synthetic construct
  source 1..51: mol_type = other DNA
cgtcggtcctatggtgctagtgggaaacaagtgtgatttgccagaccgacg

SEQ ID NO: 287 - DNA, 51 bp, synthetic construct
  source 1..51: mol_type = other DNA
cgtcggtcgagcagattaagcgagtaaaagactcggatgatgtgaccgacg

SEQ ID NO: 288 - DNA, 53 bp, synthetic construct
  source 1..53: mol_type = other DNA
cgtcggtcggcttcctctgtgtatttgccatcaataatagcaagtgaccgacg

SEQ ID NO: 289 - DNA, 51 bp, synthetic construct
  source 1..51: mol_type = other DNA
cgtcggtccagtgccatgagagaccaatacatgaggacaggcggaccgacg

SEQ ID NO: 290 - DNA, 51 bp, synthetic construct
  source 1..51: mol_type = other DNA
cgtcggtctgttggacatactggatacagctggacaagaagaggaccgacg

SEQ ID NO: 291 - DNA, 56 bp, synthetic construct
  source 1..56: mol_type = other DNA
cgtcggtcattcttacagaaaacaagtggttatagatggtgaaacctggaccgacg

SEQ ID NO: 292 - DNA, 51 bp, synthetic construct
  source 1..51: mol_type = other DNA
cgtcggtctccctccctgcccccttaccctccacacccccagggaccgacg

SEQ ID NO: 293 - DNA, 51 bp, synthetic construct
  source 1..51: mol_type = other DNA
cgtcggtcgatcccaccatagaggtgaggcccagtggtagcccgaccgacg

SEQ ID NO: 294 - DNA, 54 bp, synthetic construct
  source 1..54: mol_type = other DNA
cgtcggtcgacaatccagctaatccagaaccactttgtagatgaatgaccgacg

SEQ ID NO: 295 - DNA, 51 bp, synthetic construct
  source 1..51: mol_type = other DNA
cgtcggtctggtggttggagcaggtggtgttgggaaaagcgcagaccgacg

SEQ ID NO: 296 - DNA, 51 bp, synthetic construct
  source 1..51: mol_type = other DNA
cgtcggtcggttcttgctggtgtgaaatgactgagtacaaactgaccgacg

SEQ ID NO: 297 - DNA, 56 bp, synthetic construct
  source 1..56: mol_type = other DNA
cgtcggtctcagcaaagacaagacaggtaagtaacactgaaataaatagaccgacg

SEQ ID NO: 298 - DNA, 56 bp, synthetic construct
  source 1..56: mol_type = other DNA
cgtcggtcggacttagcaagaagttatggaattccttttattgaaacagaccgacg

SEQ ID NO: 299 - DNA, 51 bp, synthetic construct
  source 1..51: mol_type = other DNA
cgtcggtcttgccttctagaacagtagacacaaaacaggctcagaccgacg

SEQ ID NO: 300 - DNA, 55 bp, synthetic construct
  source 1..55: mol_type = other DNA
cgtcggtcctgaagatgtacctatggtcctagtaggaaataaatgtggaccgacg

SEQ ID NO: 301 - DNA, 56 bp, synthetic construct
  source 1..56: mol_type = other DNA
cgtcggtcttttttctttcccagagaacaaattaaaagagttaaggacgaccgacg

SEQ ID NO: 302 - DNA, 56 bp, synthetic construct
  source 1..56: mol_type = other DNA
cgtcggtcttgaaagatatttgtgttactaatgactgtgctataacttgaccgacg

SEQ ID NO: 303 - DNA, 56 bp, synthetic construct
  source 1..56: mol_type = other DNA
cgtcggtcggggagggctttctttgtgtatttgccataaataatactagaccgacg

SEQ ID NO: 304 - DNA, 51 bp, synthetic construct
  source 1..51: mol_type = other DNA
cgtcggtcagtacagtgcaatgagggaccagtacatgaggactgaccgacg

SEQ ID NO: 305 - DNA, 51 bp, synthetic construct
  source 1..51: mol_type = other DNA
cgtcggtctgtctcttggatattctcgacacagcaggtcaagagaccgacg

SEQ ID NO: 306 - DNA, 54 bp, synthetic construct
  source 1..54: mol_type = other DNA
cgtcggtcggattcctacaggaagcaagtagtaattgatggagaaagaccgacg

SEQ ID NO: 307 - DNA, 51 bp, synthetic construct
  source 1..51: mol_type = other DNA
cgtcggtcgcactgtaataatccagactgtgtttctcccttctgaccgacg

SEQ ID NO: 308 - DNA, 56 bp, synthetic construct
  source 1..56: mol_type = other DNA
cgtcggtccattttgtggacgaatatgatccaacaatagaggtaaatcgaccgacg

SEQ ID NO: 309 - DNA, 51 bp, synthetic construct
  source 1..51: mol_type = other DNA
cgtcggtcgcaagagtgccttgacgatacagctaattcagaatgaccgacg

SEQ ID NO: 310 - DNA, 51 bp, synthetic construct
  source 1..51: mol_type = other DNA
cgtcggtcgaatataaacttgtggtagttggagctggtggcgtgaccgacg

SEQ ID NO: 311 - DNA, 56 bp, synthetic construct
  source 1..56: mol_type = other DNA
cgtcggtcacattttcattatttttattataaggcctgctgaaaatgagaccgacg

SEQ ID NO: 312 - DNA, 55 bp, synthetic construct
  source 1..55: mol_type = other DNA
cgtcggtcgtgacagctccatttcttctaaaatagtccattggaaaggaccgacg

SEQ ID NO: 313 - DNA, 53 bp, synthetic construct
  source 1..53: mol_type = other DNA
cgtcggtcggtcatagtaatcaccagtgttctgaatcttgatgtggaccgacg

SEQ ID NO: 314 - DNA, 51 bp, synthetic construct
  source 1..51: mol_type = other DNA
cgtcggtcaactcagccaaagtggcaaatttctcccctccatagaccgacg

SEQ ID NO: 315 - DNA, 54 bp, synthetic construct
  source 1..54: mol_type = other DNA
cgtcggtcctcttttaattgcccgtgatgttccatgtaatactggagaccgacg

SEQ ID NO: 316 - DNA, 55 bp, synthetic construct
  source 1..55: mol_type = other DNA
cgtcggtccagttcagaggatatttaagctcaatgacatctccattcgaccgacg

SEQ ID NO: 317 - DNA, 51 bp, synthetic construct
  source 1..51: mol_type = other DNA
cgtcggtctcgcagtcaacacctacgaaggaaacatcatgaaggaccgacg

SEQ ID NO: 318 - DNA, 51 bp, synthetic construct
  source 1..51: mol_type = other DNA
cgtcggtcagaccgcaccatctggatggttttgggaacgtcaagaccgacg

SEQ ID NO: 319 - DNA, 54 bp, synthetic construct
  source 1..54: mol_type = other DNA
cgtcggtccaatataatgctggaccgccatatagataaatcggtacgaccgacg

SEQ ID NO: 320 - DNA, 51 bp, synthetic construct
  source 1..51: mol_type = other DNA
cgtcggtcggtacctgctcttcttcaatcctgcgctgtagtgtgaccgacg

SEQ ID NO: 321 - DNA, 51 bp, synthetic construct
  source 1..51: mol_type = other DNA
cgtcggtcgcaagagaatgagaatccgcatgccagccctcagggaccgacg

SEQ ID NO: 322 - DNA, 51 bp, synthetic construct
  source 1..51: mol_type = other DNA
cgtcggtcgtcaggggcaatgtgaggctgctatttcctacttagaccgacg

SEQ ID NO: 323 - DNA, 52 bp, synthetic construct
  source 1..52: mol_type = other DNA
cgtcggtcgattggctcgagatatcatgagtgattccaactatggaccgacg

SEQ ID NO: 324 - DNA, 51 bp, synthetic construct
  source 1..51: mol_type = other DNA
cgtcggtcgtcacccacgggaaagtggtgaagatatgtgacttgaccgacg

SEQ ID NO: 325 - DNA, 51 bp, synthetic construct
  source 1..51: mol_type = other DNA
cgtcggtcgtgtgttcacagagacctggccgccaggaacgtgcgaccgacg

SEQ ID NO: 326 - DNA, 51 bp, synthetic construct
  source 1..51: mol_type = other DNA
cgtcggtccctgctgggggcgtgcacactgtcaggtaacccacgaccgacg

SEQ ID NO: 327 - DNA, 51 bp, synthetic construct
  source 1..51: mol_type = other DNA
cgtcggtctgatgacccagctgggaagccacgagaatattgtggaccgacg

SEQ ID NO: 328 - DNA, 51 bp, synthetic construct
  source 1..51: mol_type = other DNA
cgtcggtcagctctgaaagagaggcactcatgtcagaactcaagaccgacg

SEQ ID NO: 329 - DNA, 56 bp, synthetic construct
  source 1..56: mol_type = other DNA
cgtcggtctttacatttttaatgctcctttctttgacagaaaaagcaggaccgacg

SEQ ID NO: 330 - DNA, 56 bp, synthetic construct
  source 1..56: mol_type = other DNA
cgtcggtcccaagagaaaatttagagtttggtaagaatggaatgtgccgaccgacg

SEQ ID NO: 331 - DNA, 56 bp, synthetic construct
  source 1..56: mol_type = other DNA
cgtcggtctgatttcagagaatatgaatatgatctcaaatgggagtttgaccgacg

SEQ ID NO: 332 - DNA, 51 bp, synthetic construct
  source 1..51: mol_type = other DNA
cgtcggtcgtgaccggctcctcagataatgagtacttctacgtgaccgacg

SEQ ID NO: 333 - DNA, 51 bp, synthetic construct
  source 1..51: mol_type = other DNA
cgtcggtcgcaatttaggtatgaaagccagctacagatggtacgaccgacg

SEQ ID NO: 334 - DNA, 52 bp, synthetic construct
  source 1..52: mol_type = other DNA
cgtcggtcctggaagaagtgttcagacaagtctcccaagtaatagaccgacg

SEQ ID NO: 335 - DNA, 51 bp, synthetic construct
  source 1..51: mol_type = other DNA
cgtcggtccctgtttctcggatggatacccattaccatcttgggaccgacg

SEQ ID NO: 336 - DNA, 51 bp, synthetic construct
  source 1..51: mol_type = other DNA
cgtcggtccctcaagtgctcgcagaagcatcggcaagtcaggcgaccgacg

SEQ ID NO: 337 - DNA, 53 bp, synthetic construct
  source 1..53: mol_type = other DNA
cgtcggtcccagtgagcttatttcacacgttcttttctatagggagaccgacg

SEQ ID NO: 338 - DNA, 51 bp, synthetic construct
  source 1..51: mol_type = other DNA
cgtcggtccatggcgaccaggtaggccagggtggagaggggatgaccgacg

SEQ ID NO: 339 - DNA, 51 bp, synthetic construct
  source 1..51: mol_type = other DNA
cgtcggtctggctggaccaagcccatcaccattggcaggcacggaccgacg

SEQ ID NO: 340 - DNA, 51 bp, synthetic construct
  source 1..51: mol_type = other DNA
cgtcggtcagcccatcatctgcaaaaacatcccacgcctagtcgaccgacg

SEQ ID NO: 341 - DNA, 51 bp, synthetic construct
  source 1..51: mol_type = other DNA
cgtcggtcactatccggaacatcctgggggggactgtcttccggaccgacg

SEQ ID NO: 342 - DNA, 51 bp, synthetic construct
  source 1..51: mol_type = other DNA
cgtcggtcgttcaagctgaagaagatgtggaaaagtcccaatggaccgacg

SEQ ID NO: 343 - DNA, 51 bp, synthetic construct
  source 1..51: mol_type = other DNA
cgtcggtcaggggggagcagggctcactccaggtgagtgacctgaccgacg

SEQ ID NO: 344 - DNA, 51 bp, synthetic construct
  source 1..51: mol_type = other DNA
cgtcggtcccttggaactcaaggatgcccaggctgggaaggaggaccgacg

SEQ ID NO: 345 - DNA, 51 bp, synthetic construct
  source 1..51: mol_type = other DNA
cgtcggtccgtgagcgcttcgagatgttccgagagctgaatgagaccgacg

SEQ ID NO: 346 - DNA, 51 bp, synthetic construct
  source 1..51: mol_type = other DNA
cgtcggtctacttctccccctcctctgttgctgcagatccgtggaccgacg

SEQ ID NO: 347 - DNA, 51 bp, synthetic construct
  source 1..51: mol_type = other DNA
cgtcggtcgggagcctcaccacgagctgcccccagggagcactgaccgacg

SEQ ID NO: 348 - DNA, 51 bp, synthetic construct
  source 1..51: mol_type = other DNA
cgtcggtcgaccggcgcacagaggaagagaatctccgcaagaagaccgacg

SEQ ID NO: 349 - DNA, 51 bp, synthetic construct
  source 1..51: mol_type = other DNA
cgtcggtccagctttgaggtgcgtgtttgtgcctgtcctgggagaccgacg

SEQ ID NO: 350 - DNA, 51 bp, synthetic construct
  source 1..51: mol_type = other DNA
cgtcggtcttcctatcctgagtagtggtaatctactgggacgggaccgacg

SEQ ID NO: 351 - DNA, 51 bp, synthetic construct
  source 1..51: mol_type = other DNA
cgtcggtccaccatcatcacactggaagactccaggtcaggaggaccgacg

SEQ ID NO: 352 - DNA, 51 bp, synthetic construct
  source 1..51: mol_type = other DNA
cgtcggtcgttcctgcatgggcggcatgaaccggaggcccatcgaccgacg

SEQ ID NO: 353 - DNA, 51 bp, synthetic construct
  source 1..51: mol_type = other DNA
cgtcggtcgactgtaccaccatccactacaactacatgtgtaagaccgacg

SEQ ID NO: 354 - DNA, 51 bp, synthetic construct
  source 1..51: mol_type = other DNA
cgtcggtcctcatcttgggcctgtgttatctcctaggttggctgaccgacg

SEQ ID NO: 355 - DNA, 51 bp, synthetic construct
  source 1..51: mol_type = other DNA
cgtcggtcgtgtggtggtgccctatgagccgcctgaggtctgggaccgacg

SEQ ID NO: 356 - DNA, 53 bp, synthetic construct
  source 1..53: mol_type = other DNA
cgtcggtcgtgtggagtatttggatgacagaaacacttttcgacagaccgacg

SEQ ID NO: 357 - DNA, 51 bp, synthetic construct
  source 1..51: mol_type = other DNA
cgtcggtccctcctcagcatcttatccgagtggaaggaaatttgaccgacg

SEQ ID NO: 358 - DNA, 51 bp, synthetic construct
  source 1..51: mol_type = other DNA
cgtcggtcgcctctgattcctcactgattgctcttaggtctgggaccgacg

SEQ ID NO: 359 - DNA, 51 bp, synthetic construct
  source 1..51: mol_type = other DNA
cgtcggtcgctcagatagcgatggtgagcagctggggctggaggaccgacg

SEQ ID NO: 360 - DNA, 51 bp, synthetic construct
  source 1..51: mol_type = other DNA
cgtcggtcacggaggttgtgaggcgctgcccccaccatgagcggaccgacg

SEQ ID NO: 361 - DNA, 51 bp, synthetic construct
  source 1..51: mol_type = other DNA
cgtcggtcccgcgccatggccatctacaagcagtcacagcacagaccgacg

SEQ ID NO: 362 - DNA, 51 bp, synthetic construct
  source 1..51: mol_type = other DNA
cgtcggtctgtgggttgattccacacccccgcccggcacccgcgaccgacg

SEQ ID NO: 363 - DNA, 51 bp, synthetic construct
  source 1..51: mol_type = other DNA
cgtcggtcatgttttgccaactggccaagacctgccctgtgcagaccgacg

SEQ ID NO: 364 - DNA, 51 bp, synthetic construct
  source 1..51: mol_type = other DNA
cgtcggtccttcctcttcctacagtactcccctgccctcaacagaccgacg

SEQ ID NO: 365 - DNA, 51 bp, synthetic construct
  source 1..51: mol_type = other DNA
cgtcggtcatctgttcacttgtgccctgactttcaactctgtcgaccgacg

SEQ ID NO: 366 - DNA, 51 bp, synthetic construct
  source 1..51: mol_type = other DNA
cgtcggtcgggcagctacggtttccgtctgggcttcttgcattgaccgacg

SEQ ID NO: 367 - DNA, 51 bp, synthetic construct
  source 1..51: mol_type = other DNA
cgtcggtcccctgtcatcttctgtcccttcccagaaaacctacgaccgacg

SEQ ID NO: 368 - DNA, 51 bp, synthetic construct
  source 1..51: mol_type = other DNA
cgtcggtccctacaccggcggcccctgcaccagccccctcctggaccgacg

SEQ ID NO: 369 - DNA, 51 bp, synthetic construct
  source 1..51: mol_type = other DNA
cgtcggtcagaggctgctccccccgtggcccctgcaccagcaggaccgacg

SEQ ID NO: 370 - DNA, 51 bp, synthetic construct
  source 1..51: mol_type = other DNA
cgtcggtcctgaagacccaggtccagatgaagctcccagaatggaccgacg

SEQ ID NO: 371 - DNA, 51 bp, synthetic construct
  source 1..51: mol_type = other DNA
cgtcggtccctatggaaactgtgagtggatccattggaagggcgaccgacg

SEQ ID NO: 372 - DNA, 51 bp, synthetic construct
  source 1..51: mol_type = other DNA
cgtcggtcgcgtcgagccccctctgagtcaggaaacattttcagaccgacg

SEQ ID NO: 373 - DNA, 51 bp, synthetic construct
  source 1..51: mol_type = other DNA
cgtcggtccgggtcactgccatggaggagccgcagtcagatccgaccgacg

SEQ ID NO: 374 - DNA, 51 bp, synthetic construct
  source 1..51: mol_type = other DNA
cgtcggtctccccacttttcctcttgcagcagccagactgcctgaccgacg

SEQ ID NO: 375 - DNA, 53 bp, synthetic construct
  source 1..53: mol_type = other DNA
cgtcggtcgcttatggggatcaagtaagtcatgttggcaataatggaccgacg

SEQ ID NO: 376 - DNA, 51 bp, synthetic construct
  source 1..51: mol_type = other DNA
cgtcggtcgagtggatgggtaaaacctatcatcataggtcgtcgaccgacg

SEQ ID NO: 377 - DNA, 51 bp, synthetic construct
  source 1..51: mol_type = other DNA
cgtcggtcgagaagccattatctgcaaaaatatcccccggcttgaccgacg

SEQ ID NO: 378 - DNA, 51 bp, synthetic construct
  source 1..51: mol_type = other DNA
cgtcggtcggcaccatacgaaatattctgggtggcacggtcttgaccgacg

SEQ ID NO: 379 - DNA, 56 bp, synthetic construct
  source 1..56: mol_type = other DNA
cgtcggtcgttgaggagttcaagttgaaacaaatgtggaaatcaccaagaccgacg